European Patent Application EP 4 137 507 A1, published February 22, 2023. Title: Recombinant fusion protein for preventing or treating fibrosis disease. Applicant: Korea University Research and Buisness Foundation. The sequence listing filed with the application follows.

SEQUENCE LISTING (14 sequences)

SEQ ID NO: 1 - protein, 391 aa, Artificial Sequence
  fusion protein 1_varient
  VARIANT (316): X is one of valine, alanine, and glycine
  VARIANT (390): X is alanine or glycine
MKWVWALLLLAAWAAAERDCRVSSFRVKENFDKARFSGTWYAMAKKDPEGLFLQDNIVAEFSVDETGQMSATAKGRVRLLNNWDVCADMVGTFTDTEDPAKFKMKYWGVASFLQKGNDDHWIVDTDYDTYAVQYSCRLLNLDGTCADSYSFVFSRDPNGLPPEAQKIVRQRQEELCLARQYRLIVHNGYCDGRLVEEPQNLIKQNCELFEQLGEYKFQNALLVRYTKKVPEVSTPTLVEVSRNLGKVGSKCCKHPEAKRMPCAEDYLSVVLNQLCVLHEKTPVSDRVTKCCTESLVNRRPCFSALEVDETYVPKEXNAETFTFHADICTLSEKERQIKKQTALVELVKHKPKATKEQLKAVMDDFAAFVEKCCKADDKETCFAEEGKKLXA

SEQ ID NO: 2 - protein, 392 aa, Artificial Sequence
  fusion protein 2_varient
  VARIANT (141): X is one of valine, alanine, and glycine
  VARIANT (215): X is alanine or glycine
MKWVTFISLLFLFSSAYSLVEEPQNLIKQNCELFEQLGEYKFQNALLVRYTKKVPEVSTPTLVEVSRNLGKVGSKCCKHPEAKRMPCAEDYLSVVLNQLCVLHEKTPVSDRVTKCCTESLVNRRPCFSALEVDETYVPKEXNAETFTFHADICTLSEKERQIKKQTALVELVKHKPKATKEQLKAVMDDFAAFVEKCCKADDKETCFAEEGKKLXAERDCRVSSFRVKENFDKARFSGTWYAMAKKDPEGLFLQDNIVAEFSVDETGQMSATAKGRVRLLNNWDVCADMVGTFTDTEDPAKFKMKYWGVASFLQKGNDDHWIVDTDYDTYAVQYSCRLLNLDGTCADSYSFVFSRDPNGLPPEAQKIVRQRQEELCLARQYRLIVHNGYCDG

SEQ ID NO: 3 - protein, 391 aa, Artificial Sequence
  fusion protein 1
MKWVWALLLLAAWAAAERDCRVSSFRVKENFDKARFSGTWYAMAKKDPEGLFLQDNIVAEFSVDETGQMSATAKGRVRLLNNWDVCADMVGTFTDTEDPAKFKMKYWGVASFLQKGNDDHWIVDTDYDTYAVQYSCRLLNLDGTCADSYSFVFSRDPNGLPPEAQKIVRQRQEELCLARQYRLIVHNGYCDGRLVEEPQNLIKQNCELFEQLGEYKFQNALLVRYTKKVPEVSTPTLVEVSRNLGKVGSKCCKHPEAKRMPCAEDYLSVVLNQLCVLHEKTPVSDRVTKCCTESLVNRRPCFSALEVDETYVPKEVNAETFTFHADICTLSEKERQIKKQTALVELVKHKPKATKEQLKAVMDDFAAFVEKCCKADDKETCFAEEGKKLAA

SEQ ID NO: 4 - protein, 392 aa, Artificial Sequence
  fusion protein 2
MKWVTFISLLFLFSSAYSLVEEPQNLIKQNCELFEQLGEYKFQNALLVRYTKKVPEVSTPTLVEVSRNLGKVGSKCCKHPEAKRMPCAEDYLSVVLNQLCVLHEKTPVSDRVTKCCTESLVNRRPCFSALEVDETYVPKEVNAETFTFHADICTLSEKERQIKKQTALVELVKHKPKATKEQLKAVMDDFAAFVEKCCKADDKETCFAEEGKKLAAERDCRVSSFRVKENFDKARFSGTWYAMAKKDPEGLFLQDNIVAEFSVDETGQMSATAKGRVRLLNNWDVCADMVGTFTDTEDPAKFKMKYWGVASFLQKGNDDHWIVDTDYDTYAVQYSCRLLNLDGTCADSYSFVFSRDPNGLPPEAQKIVRQRQEELCLARQYRLIVHNGYCDG

SEQ ID NO: 5 - protein, 395 aa, Artificial Sequence
  fusion protein 3
MKWVWALLLLAAWAAAERDCRVSSFRVKENFDKARFSGTWYAMAKKDPEGLFLQDNIVAEFSVDETGQMSATAKGRVRLLNNWDVCADMVGTFTDTEDPAKFKMKYWGVASFLQKGNDDHWIVDTDYDTYAVQYSCRLLNLDGTCADSYSFVFSRDPNGLPPEAQKIVRQRQEELCLARQYRLIVHNGYCDGRLVEEPQNLIKQNCELFEQLGEYKFQNALLVRYTKKVPEVSTPTLVEVSRNLGKVGSKCCKHPEAKRMPCAEDYLSVVLNQLCVLHEKTPVSDRVTKCCTESLVNRRPCFSALEVDDNPNLPRLVRPEVDVMCTAFHDNEETFLKKYLYEIARRHPYFYAPELLFFAKRYKAAFTECCQAADKAACLLPKLDELRDEGKASSA

SEQ ID NO: 6 - protein, 392 aa, Artificial Sequence
  fusion protein 4
MKWVWALLLLAAWAAAERDCRVSSFRVKENFDKARFSGTWYAMAKKDPEGLFLQDNIVAEFSVDETGQMSATAKGRVRLLNNWDVCADMVGTFTDTEDPAKFKMKYWGVASFLQKGNDDHWIVDTDYDTYAVQYSCRLLNLDGTCADSYSFVFSRDPNGLPPEAQKIVRQRQEELCLARQYRLIVHNGYCDGRLVEEPQNLIKQNCELFEQLGEYKFQNALLVRYTKKVPEVSTPTLVEVSRNLGKVGSKCCKHPEAKRMPCAEDYLSVVLNQLCVLHEKTPVSDRVTKCCTESLVNRRPCFSALEVPNLPRLVRPEVDVMCTAFHDNEETFLKKYLYEIARRHPYFYAPELLFFAKRYKAAFTECCQAADKAACLLPKLDELRDEGKASSA

SEQ ID NO: 7 - protein, 396 aa, Artificial Sequence
  fusion protein 5
MKWVTFISLLFLFSSAYSLVEEPQNLIKQNCELFEQLGEYKFQNALLVRYTKKVPEVSTPTLVEVSRNLGKVGSKCCKHPEAKRMPCAEDYLSVVLNQLCVLHEKTPVSDRVTKCCTESLVNRRPCFSALEVDDNPNLPRLVRPEVDVMCTAFHDNEETFLKKYLYEIARRHPYFYAPELLFFAKRYKAAFTECCQAADKAACLLPKLDELRDEGKASSAERDCRVSSFRVKENFDKARFSGTWYAMAKKDPEGLFLQDNIVAEFSVDETGQMSATAKGRVRLLNNWDVCADMVGTFTDTEDPAKFKMKYWGVASFLQKGNDDHWIVDTDYDTYAVQYSCRLLNLDGTCADSYSFVFSRDPNGLPPEAQKIVRQRQEELCLARQYRLIVHNGYCDG

SEQ ID NO: 8 - protein, 393 aa, Artificial Sequence
  fusion protein 6
MKWVTFISLLFLFSSAYSLVEEPQNLIKQNCELFEQLGEYKFQNALLVRYTKKVPEVSTPTLVEVSRNLGKVGSKCCKHPEAKRMPCAEDYLSVVLNQLCVLHEKTPVSDRVTKCCTESLVNRRPCFSALEVPNLPRLVRPEVDVMCTAFHDNEETFLKKYLYEIARRHPYFYAPELLFFAKRYKAAFTECCQAADKAACLLPKLDELRDEGKASSAERDCRVSSFRVKENFDKARFSGTWYAMAKKDPEGLFLQDNIVAEFSVDETGQMSATAKGRVRLLNNWDVCADMVGTFTDTEDPAKFKMKYWGVASFLQKGNDDHWIVDTDYDTYAVQYSCRLLNLDGTCADSYSFVFSRDPNGLPPEAQKIVRQRQEELCLARQYRLIVHNGYCDG

SEQ ID NO: 9 - DNA, 1173 bp, Artificial Sequence
  DNA encoding fusion protein 1
atgaagtgggtgtgggctctgctgctgctggctgcttgggccgctgccgagagagattgccgcgtgtccagcttcagagtgaaggagaacttcgacaaggcccgcttttccggcacctggtacgctatggccaagaaggaccccgagggcctgttcctgcaggacaatatcgtggctgagtttagcgtggatgagacaggccagatgtctgctaccgccaagggcagagtgcgcctgctgaacaattgggacgtgtgcgctgacatggtgggcaccttcacagataccgaggacccagccaagtttaagatgaagtattggggcgtggctagctttctgcagaagggcaacgacgatcactggatcgtggacacagattacgacacctatgccgtgcagtacagctgcagactgctgaacctggatggcacatgtgctgactcttattccttcgtgttttctcgcgatccaaatggcctgccccctgaggcccagaagatcgtgaggcagaggcaggaggagctgtgcctggctaggcagtaccggctgatcgtgcataatggctattgtgacggcaggctggtggaggagccccagaacctgatcaagcagaattgcgagctgttcgagcagctgggcgagtacaagtttcagaacgccctgctggtgcggtataccaagaaggtgccagaggtgtccacacccaccctggtggaggtgagcaggaatctgggcaaggtcggctctaagtgctgtaagcaccctgaggctaagcggatgccatgcgccgaggattacctgtctgtggtgctgaaccagctgtgcgtgctgcatgagaagacacccgtgtccgacagagtgacaaagtgctgtaccgagtccctggtgaacaggcggccctgcttcagcgccctggaggtggatgagacctatgtgcctaaggaggttaatgctgagacattcacctttcacgccgacatctgtacactgtctgagaaggagcgccagatcaagaagcagaccgctctggtggagctggtgaagcataagcctaaggctacaaaggagcagctgaaggccgtgatggacgatttcgctgcctttgtggagaagtgctgtaaggctgacgataaggagacctgtttcgccgaggagggcaagaagctggcggct

SEQ ID NO: 10 - DNA, 1176 bp, Artificial Sequence
  DNA encoding fusion protein 2
atgaagtgggtgacattcatcagcctgctgttcctgttctcctccgcctactctctggtggaggagccccagaacctgatcaagcagaattgcgagctgttcgagcagctgggcgagtacaagtttcagaacgccctgctggtgaggtataccaagaaggtgccagaggtgtccacccccacactggtggaggtgagcaggaatctgggcaaggtcggctctaagtgctgtaagcaccctgaggccaagcggatgccatgcgctgaggattacctgtccgtggtgctgaaccagctgtgcgtgctgcatgagaagacacctgtgagcgacagggtgacaaagtgctgtaccgagtctctggtgaacaggcggccctgcttctccgctctggaggtggatgagacctatgtgcctaaggaggttaatgccgagaccttcacatttcacgctgacatctgtacactgtccgagaaggagagacagatcaagaagcagaccgccctggtggagctggtgaagcataagccaaaggccacaaaggagcagctgaaggctgtgatggacgatttcgccgcttttgtggagaagtgctgtaaggccgacgataaggagacctgcttcgctgaggagggcaagaagctggcggccgagagagattgtcgcgtgtcttcctttagagtgaaggagaacttcgacaaggctcgctttagcggcacatggtacgctatggccaagaaggaccccgagggcctgttcctgcaggacaatatcgtggccgagttttccgtggatgagacaggccagatgagcgccaccgctaagggaagagtgcgcctgctgaacaattgggacgtgtgcgccgacatggtgggcaccttcacagataccgaggaccccgctaagtttaagatgaagtattggggcgtggcctcttttctgcagaagggcaacgacgatcactggatcgtggacacagattacgacacctatgctgtgcagtactcttgcagactgctgaacctggatggcacctgtgccgacagctattctttcgtgttttcccgcgatcctaatggcctgccccctgaggctcagaagatcgtgaggcagaggcaggaggagctgtgcctggccaggcagtaccggctgatcgtgcataatggctattgtgacggc

SEQ ID NO: 11 - DNA, 1185 bp, Artificial Sequence
  DNA encoding fusion protein 3
atgaagtgggtgtgggctctgctgctgctggctgcttgggccgctgccgagagagattgccgcgtgtccagcttcagagtgaaggagaacttcgacaaggcccgcttttccggcacctggtacgctatggccaagaaggaccccgagggcctgttcctgcaggacaatatcgtggctgagtttagcgtggatgagacaggccagatgtctgctaccgccaagggcagagtgcgcctgctgaacaattgggacgtgtgcgctgacatggtgggcaccttcacagataccgaggacccagccaagtttaagatgaagtattggggcgtggctagctttctgcagaagggcaacgacgatcactggatcgtggacacagattacgacacctatgccgtgcagtacagctgcagactgctgaacctggatggcacatgtgctgactcttattccttcgtgttttctcgcgatccaaatggcctgccccctgaggcccagaagatcgtgaggcagaggcaggaggagctgtgcctggctaggcagtaccggctgatcgtgcataatggctattgtgacggcaggctggtggaggagccccagaacctgatcaagcagaattgcgagctgttcgagcagctgggcgagtacaagtttcagaacgccctgctggtgcggtataccaagaaggtgccagaggtgtccacacccaccctggtggaggtgagcaggaatctgggcaaggtcggctctaagtgctgtaagcaccctgaggctaagcggatgccatgcgccgaggattacctgtctgtggtgctgaaccagctgtgcgtgctgcatgagaagacacccgtgtccgacagagtgacaaagtgctgtaccgagtccctggtgaacaggcggccctgcttcagcgccctggaggtggacgataacccaaatctgcccagactggtgcgcccagaggtggatgtgatgtgcacagctttccacgacaatgaggagacctttctgaagaagtacctgtatgagatcgccagacgccatccctacttttatgctcctgagctgctgttctttgccaagcggtacaaggctgccttcacagagtgctgtcaggctgctgacaaggctgcttgcctgctgccaaagctggatgagctgagggacgagggcaaggcttcttccgcc

SEQ ID NO: 12 - DNA, 1176 bp, Artificial Sequence
  DNA encoding fusion protein 4
atgaagtgggtgtgggctctgctgctgctggctgcttgggccgctgccgagagagattgccgcgtgtccagcttcagagtgaaggagaacttcgacaaggcccgcttttccggcacctggtacgctatggccaagaaggaccccgagggcctgttcctgcaggacaatatcgtggctgagtttagcgtggatgagacaggccagatgtctgctaccgccaagggcagagtgcgcctgctgaacaattgggacgtgtgcgctgacatggtgggcaccttcacagataccgaggacccagccaagtttaagatgaagtattggggcgtggctagctttctgcagaagggcaacgacgatcactggatcgtggacacagattacgacacctatgccgtgcagtacagctgcagactgctgaacctggatggcacatgtgctgactcttattccttcgtgttttctcgcgatccaaatggcctgccccctgaggcccagaagatcgtgaggcagaggcaggaggagctgtgcctggctaggcagtaccggctgatcgtgcataatggctattgtgacggcaggctggtggaggagccccagaacctgatcaagcagaattgcgagctgttcgagcagctgggcgagtacaagtttcagaacgccctgctggtgcggtataccaagaaggtgccagaggtgtccacacccaccctggtggaggtgagcaggaatctgggcaaggtcggctctaagtgctgtaagcaccctgaggctaagcggatgccatgcgccgaggattacctgtctgtggtgctgaaccagctgtgcgtgctgcatgagaagacacccgtgtccgacagagtgacaaagtgctgtaccgagtccctggtgaacaggcggccctgcttcagcgccctggaggtgccaaatctgcccagactggtgcgcccagaggtggatgtgatgtgcacagctttccacgacaatgaggagacctttctgaagaagtacctgtatgagatcgccagacgccatccctacttttatgctcctgagctgctgttctttgccaagcggtacaaggctgccttcacagagtgctgtcaggctgctgacaaggctgcttgcctgctgccaaagctggatgagctgagggacgagggcaaggcttcttccgcc

SEQ ID NO: 13 - DNA, 1188 bp, Artificial Sequence
  DNA encoding fusion protein 5
atgaagtgggtgacattcatcagcctgctgttcctgttctcctccgcctactctctggtggaggagccccagaacctgatcaagcagaattgcgagctgttcgagcagctgggcgagtacaagtttcagaacgccctgctggtgaggtataccaagaaggtgccagaggtgtccacccccacactggtggaggtgagcaggaatctgggcaaggtcggctctaagtgctgtaagcaccctgaggccaagcggatgccatgcgctgaggattacctgtccgtggtgctgaaccagctgtgcgtgctgcatgagaagacacctgtgagcgacagggtgacaaagtgctgtaccgagtctctggtgaacaggcggccctgcttctccgctctggaggtggacgataacccaaatctgcccagactggtgcgcccagaggtggatgtgatgtgcacagctttccacgacaatgaggagacctttctgaagaagtacctgtatgagatcgccagacgccatccctacttttatgctcctgagctgctgttctttgccaagcggtacaaggctgccttcacagagtgctgtcaggctgctgacaaggctgcttgcctgctgccaaagctggatgagctgagggacgagggcaaggcttcttccgccgagagagattgccgcgtgtccagcttcagagtgaaggagaacttcgacaaggcccgcttttccggcacctggtacgctatggccaagaaggaccccgagggcctgttcctgcaggacaatatcgtggctgagtttagcgtggatgagacaggccagatgtctgctaccgccaagggcagagtgcgcctgctgaacaattgggacgtgtgcgctgacatggtgggcaccttcacagataccgaggacccagccaagtttaagatgaagtattggggcgtggctagctttctgcagaagggcaacgacgatcactggatcgtggacacagattacgacacctatgccgtgcagtacagctgcagactgctgaacctggatggcacatgtgctgactcttattccttcgtgttttctcgcgatccaaatggcctgccccctgaggcccagaagatcgtgaggcagaggcaggaggagctgtgcctggctaggcagtaccggctgatcgtgcataatggctattgtgacggc

SEQ ID NO: 14 - DNA, 1179 bp, Artificial Sequence
  DNA encoding fusion protein 6
atgaagtgggtgacattcatcagcctgctgttcctgttctcctccgcctactctctggtggaggagccccagaacctgatcaagcagaattgcgagctgttcgagcagctgggcgagtacaagtttcagaacgccctgctggtgaggtataccaagaaggtgccagaggtgtccacccccacactggtggaggtgagcaggaatctgggcaaggtcggctctaagtgctgtaagcaccctgaggccaagcggatgccatgcgctgaggattacctgtccgtggtgctgaaccagctgtgcgtgctgcatgagaagacacctgtgagcgacagggtgacaaagtgctgtaccgagtctctggtgaacaggcggccctgcttctccgctctggaggtgccaaatctgcccagactggtgcgcccagaggtggatgtgatgtgcacagctttccacgacaatgaggagacctttctgaagaagtacctgtatgagatcgccagacgccatccctacttttatgctcctgagctgctgttctttgccaagcggtacaaggctgccttcacagagtgctgtcaggctgctgacaaggctgcttgcctgctgccaaagctggatgagctgagggacgagggcaaggcttcttccgccgagagagattgccgcgtgtccagcttcagagtgaaggagaacttcgacaaggcccgcttttccggcacctggtacgctatggccaagaaggaccccgagggcctgttcctgcaggacaatatcgtggctgagtttagcgtggatgagacaggccagatgtctgctaccgccaagggcagagtgcgcctgctgaacaattgggacgtgtgcgctgacatggtgggcaccttcacagataccgaggacccagccaagtttaagatgaagtattggggcgtggctagctttctgcagaagggcaacgacgatcactggatcgtggacacagattacgacacctatgccgtgcagtacagctgcagactgctgaacctggatggcacatgtgctgactcttattccttcgtgttttctcgcgatccaaatggcctgccccctgaggcccagaagatcgtgaggcagaggcaggaggagctgtgcctggctaggcagtaccggctgatcgtgcataatggctattgtgacggc